European Patent Specification EP 4 229 205 B1, published May 14, 2025. Title: Nucleic acid constructs for VA RNA transcription. Applicant: F. Hoffmann-La Roche AG. The sequence listing filed with the application follows.

SEQUENCE LISTING (45 sequences)

SEQ ID NO: 1 - DNA, 13 bp, Bacteriophage P1
ataacttcgtata

SEQ ID NO: 2 - DNA, 13 bp, Bacteriophage P1
tatacgaagttat

SEQ ID NO: 3 - DNA, 8 bp, Bacteriophage P1
atgtatgc

SEQ ID NO: 4 - DNA, 8 bp, Artificial Sequence
  L3 spacer sequence
aagtctcc

SEQ ID NO: 5 - DNA, 8 bp, Artificial Sequence
  L2 inverted spacer sequence
gcatacat

SEQ ID NO: 6 - DNA, 8 bp, Artificial Sequence
  LoxFas spacer sequence
tacctttc

SEQ ID NO: 7 - DNA, 8 bp, Artificial Sequence
  Lox511 spacer sequence
atgtatac

SEQ ID NO: 8 - DNA, 8 bp, Artificial Sequence
  Lox5171 spacer sequence
atgtgtac

SEQ ID NO: 9 - DNA, 8 bp, Artificial Sequence
  Lox2272 spacer sequence
aagtatcc

SEQ ID NO: 10 - DNA, 8 bp, Artificial Sequence
  Loxm2 spacer sequence
agaaacca

SEQ ID NO: 11 - DNA, 8 bp, Artificial Sequence
  Loxm3 spacer sequence
taatacca

SEQ ID NO: 12 - DNA, 8 bp, Artificial Sequence
  Loxm7 spacer sequence
agatagaa

SEQ ID NO: 13 - DNA, 608 bp, Human cytomegalovirus
gttgacattgattattgactagttattaatagtaatcaattacggggtcattagttcatagcccatatatggagttccgcgttacataacttacggtaaatggcccgcctggctgaccgcccaacgacccccgcccattgacgtcaataatgacgtatgttcccatagtaacgccaatagggactttccattgacgtcaatgggtggagtatttacggtaaactgcccacttggcagtacatcaagtgtatcatatgccaagtacgccccctattgacgtcaatgacggtaaatggcccgcctggcattatgcccagtacatgaccttatgggactttcctacttggcagtacatctacgtattagtcatcgctattagcatggtgatgcggttttggcagtacatcaatgggcgtggatagcggtttgactcacggggatttccaagtctccaccccattgacgtcaatgggagtttgttttggcaccaaaatcaacgggactttccaaaatgtcgtaacaactccgccccattgacgcaaatgggcggtaggcgtgtacggtgggaggtctatataagcagagctccgtttagtgaacgtcagatc

SEQ ID NO: 14 - DNA, 696 bp, Human cytomegalovirus
gttgacattgattattgactagttattaatagtaatcaattacggggtcattagttcatagcccatatatggagttccgcgttacataacttacggtaaatggcccgcctggctgaccgcccaacgacccccgcccattgacgtcaataatgacgtatgttcccatagtaacgccaatagggactttccattgacgtcaatgggtggagtatttacggtaaactgcccacttggcagtacatcaagtgtatcatatgccaagtacgccccctattgacgtcaatgacggtaaatggcccgcctggcattatgcccagtacatgaccttatgggactttcctacttggcagtacatctacgtattagtcatcgctattagcatggtgatgcggttttggcagtacatcaatgggcgtggatagcggtttgactcacggggatttccaagtctccaccccattgacgtcaatgggagtttgttttggcaccaaaatcaacgggactttccaaaatgtcgtaacaactccgccccattgacgcaaatgggcggtaggcgtgtacggtgggaggtctatataagcagagctccgtttagtgaacgtcagatctagctctgggagaggagcccagcactagaagtcggcggtgtttccattcggtgatcagcactgaacacagaggaagcttgccgccacc

SEQ ID NO: 15 - DNA, 2125 bp, Human cytomegalovirus
ctgcagtgaataataaaatgtgtgtttgtccgaaatacgcgttttgagatttctgtcgccgactaaattcatgtcgcgcgatagtggtgtttatcgccgatagagatggcgatattggaaaaatcgatatttgaaaatatggcatattgaaaatgtcgccgatgtgagtttctgtgtaactgatatcgccatttttccaaaagtgatttttgggcatacgcgatatctggcgatagcgcttatatcgtttacgggggatggcgatagacgactttggtgacttgggcgattctgtgtgtcgcaaatatcgcagtttcgatataggtgacagacgatatgaggctatatcgccgatagaggcgacatcaagctggcacatggccaatgcatatcgatctatacattgaatcaatattggccattagccatattattcattggttatatagcataaatcaatattggctattggccattgcatacgttgtatccatatcataatatgtacatttatattggctcatgtccaacattaccgccatgttgacattgattattgactagttattaatagtaatcaattacggggtcattagttcatagcccatatatggagttccgcgttacataacttacggtaaatggcccgcctggctgaccgcccaacgacccccgcccattgacgtcaataatgacgtatgttcccatagtaacgccaatagggactttccattgacgtcaatgggtggagtatttacggtaaactgcccacttggcagtacatcaagtgtatcatatgccaagtacgccccctattgacgtcaatgacggtaaatggcccgcctggcattatgcccagtacatgaccttatgggactttcctacttggcagtacatctacgtattagtcatcgctattaccatggtgatgcggttttggcagtacatcaatgggcgtggatagcggtttgactcacggggatttccaagtctccaccccattgacgtcaatgggagtttgttttggcaccaaaatcaacgggactttccaaaatgtcgtaacaactccgccccattgacgcaaatgggcggtaggcgtgtacggtgggaggtctatataagcagagctcgtttagtgaaccgtcagatcgcctggagacgccatccacgctgttttgacctccatagaagacaccgggaccgatccagcctccgcggccgggaacggtgcattggaacgcggattccccgtgccaagagtgacgtaagtaccgcctatagagtctataggcccacccccttggcttcttatgcatgctatactgtttttggcttggggtctatacacccccgcttcctcatgttataggtgatggtatagcttagcctataggtgtgggttattgaccattattgaccactcccctattggtgacgatactttccattactaatccataacatggctctttgccacaactctctttattggctatatgccaatacactgtccttcagagactgacacggactctgtatttttacaggatggggtctcatttattatttacaaattcacatatacaacaccaccgtccccagtgcccgcagtttttattaaacataacgtgggatctccacgcgaatctcgggtacgtgttccggacatgggctcttctccggtagcggcggagcttctacatccgagccctgctcccatgcctccagcgactcatggtcgctcggcagctccttgctcctaacagtggaggccagacttaggcacagcacgatgcccaccaccaccagtgtgccgcacaaggccgtggcggtagggtatgtgtctgaaaatgagctcggggagcgggcttgcaccgctgacgcatttggaagacttaaggcagcggcagaagaagatgcaggcagctgagttgttgtgttctgataagagtcagaggtaactcccgttgcggtgctgttaacggtggagggcagtgtagtctgagcagtactcgttgctgccgcgcgcgccaccagacataatagctgacagactaacagactgttcctttccatgggtcttttctgcagtcaccgtccttgacacggtttaaacgccgccacc

SEQ ID NO: 16 - DNA, 218 bp, Bos taurus
ttctagttgccagccatctgttgtttgcccctcccccgtgccttccttgaccctggaaggtgccactcccactgtcctttcctaataaaatgaggaaattgcatcgcattgtctgagtaggtgtcattctattctggggggtggggtggggcaggacagcaagggggaggattgggaagacaatagcaggcatgctggggatgcggtgggctctatgg

SEQ ID NO: 17 - DNA, 73 bp, Homo sapiens
caggataatatatggtagggttcatagccagagtaacctttttttttaatttttattttattttatttttgag

SEQ ID NO: 18 - DNA, 288 bp, Simian virus 40
agtcagcaaccaggtgtggaaagtccccaggctccccagcaggcagaagtatgcaaagcatgcatctcaattagtcagcaaccatagtcccgcccctaactccgcccatcccgcccctaactccgcccagttccgcccattctccgccccatggctgactaattttttttatttatgcagaggccgaggccgcctctgcctctgagctattccagaagtagtgaggaggcttttttggaggcctaggcttttgcaaaaagctcccgggagcttgtatatccattttcg

SEQ ID NO: 19 - DNA, 129 bp, Simian virus 40
aacttgtttattgcagcttataatggttacaaataaagcaatagcatcacaaatttcacaaataaagcatttttttcaccattctagttgtggtttgtccaaactcatcaatgtatcttatcatgtctg

SEQ ID NO: 20 - DNA, 34 bp, Saccharomyces cerevisiae
gaagttcctattctctagaaagtataggaacttc

SEQ ID NO: 21 - DNA, 13 bp, Saccharomyces cerevisiae
gaagttcctattc

SEQ ID NO: 22 - DNA, 13 bp, Saccharomyces cerevisiae
gaataggaacttc

SEQ ID NO: 23 - DNA, 8 bp, Saccharomyces cerevisiae
tctagaaa

SEQ ID NO: 24 - DNA, 8 bp, Artificial Sequence
  F3 site spacer sequence
ttcaaata

SEQ ID NO: 25 - DNA, 8 bp, Artificial Sequence
  F5 site spacer sequence
ttcaaaag

SEQ ID NO: 26 - protein, 343 aa, Bacteriophage P1
MSNLLTVHQNLPALPVDATSDEVRKNLMDMFRDRQAFSEHTWKMLLSVCRSWAAWCKLNNRKWFPAEPEDVRDYLLYLQARGLAVKTIQQHLGQLNMLHRRSGLPRPSDSNAVSLVMRRIRKENVDAGERAKQALAFERTDFDQVRSLMENSDRCQDIRNLAFLGIAYNTLLRIAEIARIRVKDISRTDGGRMLIHIGRTKTLVSTAGVEKALSLGVTKLVERWISVSGVADDPNNYLFCRVRKNGVAAPSATSQLSTRALEGIFEATHRLIYGAKDDSGQRYLAWSGHSARVGAARDMARAGVSIPEIMQAGGWTNVNIVMNYIRNLDSETGAMVRLLEDGD

SEQ ID NO: 27 - RNA, 1029 nt, Bacteriophage P1
augagcaaccugcugaccgugcaccagaaccugcccgcccugcccguggacgccaccagcgacgaggugaggaagaaccugauggacauguucagggacaggcaggccuucagcgagcacaccuggaagaugcugcugagcgugugcaggagcugggccgccuggugcaagcugaacaacaggaagugguuccccgccgagcccgaggacgugagggacuaccugcuguaccugcaggccaggggccuggccgugaagaccauccagcagcaccugggccagcugaacaugcugcacaggaggagcggccugcccaggcccagcgacagcaacgccgugagccuggugaugaggaggaucaggaaggagaacguggacgccggcgagagggccaagcaggcccuggccuucgagaggaccgacuucgaccaggugaggagccugauggagaacagcgacaggugccaggacaucaggaaccuggccuuccugggcaucgccuacaacacccugcugaggaucgccgagaucgccaggaucagggugaaggacaucagcaggaccgacggcggcaggaugcugauccacaucggcaggaccaagacccuggugagcaccgccggcguggagaaggcccugagccugggcgugaccaagcugguggagagguggaucagcgugagcggcguggccgacgaccccaacaacuaccuguucugcagggugaggaagaacggcguggccgcccccagcgccaccagccagcugagcaccagggcccuggagggcaucuucgaggccacccacaggcugaucuacggcgccaaggacgacagcggccagagguaccuggccuggagcggccacagcgccagggugggcgccgccagggacauggccagggccggcgugagcauccccgagaucaugcaggccggcggcuggaccaacgugaacaucgugaugaacuacaucaggaaccuggacagcgagaccggcgccauggugaggcugcuggaggacggcgac

SEQ ID NO: 28 - DNA, 798 bp, Artificial Sequence
  green fluorescent protein encoding nucleic acid
atggtgagcaagggcgaggagctgttcaccggggtggtgcccatcctggtcgagctggacggcgacgtaaacggccacaagttcagcgtgtccggcgagggcgagggcgatgccacctacggcaagctgaccctgaagttcatctgcaccaccggcaagctgcccgtgccctggcccaccctcgtgaccaccctgacctacggcgtgcagtgcttcagccgctaccccgaccacatgaagcagcacgacttcttcaagtccgccatgcccgaaggctacgtccaggagcgcaccatcttcttcaaggacgacggcaactacaagacccgcgccgaggtgaagttcgagggcgacaccctggtgaaccgcatcgagctgaagggcatcgacttcaaggaggacggcaacatcctggggcacaagctggagtacaactacaacagccacaacgtctatatcatggccgacaagcagaagaacggcatcaaggtgaacttcaagatccgccacaacatcgaggacggcagcgtgcagctcgccgaccactaccagcagaacacccccatcggcgacggccccgtgctgctgcccgacaaccactacctgagcacccagtccgccctgagcaaagaccccaacgagaagcgcgatcacatggtcctgctggagttcgtgaccgccgccgggatcactctcggcatggacgagctgtacaagtccggactcagatctcgagctcaagcttcgaattctgcagtcgacggtaccgcgggcccgggatccaccggatctagatga

SEQ ID NO: 29 - RNA, 4 nt, Human adenovirus type 2
ccgg

SEQ ID NO: 30 - RNA, 5 nt, Human adenovirus type 2
yccgg

SEQ ID NO: 31 - RNA, 10 nt, Artificial Sequence
  VA RNA A-box consensus sequence
  misc_feature (4)..(5): n is a, c, g, or u
rrynnarygg

SEQ ID NO: 32 - RNA, 9 nt, Artificial Sequence
  VA RNA B-box consensus sequence
  misc_feature (7)..(8): n is a, c, g, or u
gwucrannc

SEQ ID NO: 33 - DNA, 225 bp, Human adenovirus type 2
cgtgcaaaaggagagcctgtaagcgggcactcttccgtggtctggtggataaattcgcaagggtatcatggcggacgaccggggttcgaaccccggatccggccgtccgccgtgatccatgcggttaccgcccgcgtgtcgaacccaggtgtgcgacgtcagacaacgggggagcgctccttttggcttccttccaggcgcggcggctgctgcgctagctttttt

SEQ ID NO: 34 - DNA, 225 bp, Human adenovirus type 2
cgtgcaaaaggagagcctgtaagcgggcactcttccgtggtctggtggataaattcgcaagggtatcatggcggacgaccgttgttcgaacaccggatccggccgtccgccgtgatccatgcggttaccgcccgcgtgtcgaacccaggtgtgcgacgtcagacaacgggggagcgctccttttggcttccttccaggcgcggcggctgctgcgctagctttttt

SEQ ID NO: 35 - DNA, 242 bp, Human adenovirus type 5
tcgttgacgctctagaccgtgcaaaaggagagcctgtaagcgggcactcttccgtggtctggtggataaattcgcaagggtatcatggcggacgaccggggttcgagccccgtatccggccgtccgccgtgatccatgcggttaccgcccgcgtgtcgaacccaggtgtgcgacgtcagacaacgggggagtgctccttttggcttccttccaggcgcggcggctgctgcgctagctttttt

SEQ ID NO: 36 - DNA, 466 bp, Human adenovirus type 5
tcgttgacgctctagaccgtgcaaaaggagagcctgtaagcgggcactcttccgtggtctggtggataaattcgcaagggtatcatggcggacgaccggggttcgagccccgtatccggccgtccgccgtgatccatgcggttaccgcccgcgtgtcgaacccaggtgtgcgacgtcagacaacgggggagtgctccttttggcttccttccaggcgcggcggctgctgcgctagcttttttggccactggccgcgcgcagcgtaagcggttaggctggaaagcgaaagcattaagtggctcgctccctgtagccggagggttattttccaagggttgagtcgcgggacccccggttcgagtctcggaccggccggactgcggcgaacgggggtttgcctccccgtcatgcaagaccccgcttgcaaattcctccggaaacagggacgagccccttttttgctttt

SEQ ID NO: 37 - DNA, 201 bp, adeno-associated virus 2
gggcactcttccgtggtctggtggataaattcgcaagggtatcatggcggacgaccggggttcgaaccccggatccggccgtccgccgtgatccatgcggttaccgcccgcgtgtcgaacccaggtgtgcgacgtcagacaacgggggagcgctccttttggcttccttccaggcgcggcggctgctgcgctagctttttt

SEQ ID NO: 38 - DNA, 201 bp, adeno-associated virus 2
gggcactcttccgtggtctggtggataaattcgcaagggtatcatggcggacgaccgttgttcgaacaccggatccggccgtccgccgtgatccatgcggttaccgcccgcgtgtcgaacccaggtgtgcgacgtcagacaacgggggagcgctccttttggcttccttccaggcgcggcggctgctgcgctagctttttt

SEQ ID NO: 39 - DNA, 465 bp, Artificial Sequence
  stuffer sequence
aaggtcgggcaggaagagggcctatttcccatgattccttcatatttgcatatacgatacaaggctgttagagagataattagaattaatttgactgtaaacacaaagatattagtacaaaatacgtgacgtagaaagtaataatttcttgggtagtttgcagttttaaaattatgttttaaaatggactatcatatgcttaccgtaacttgaaagtatttcgatttcttggctttatatatcttgtggaaaggacgaaacaccgggcactcttccgtggtctggtggataaattcgcaagggtatcatggcggacgaccggggttcgaaccccggatccggccgtccgccgtgatccatgcggttaccgcccgcgtgtcgaacccaggtgtgcgacgtcagacaacgggggagcgctccttttggcttccttccaggcgcggcggctgctgcgctagctttttt

SEQ ID NO: 40 - protein, 738 aa, Artificial Sequence
  VP1 Capsid
MAADGYLPDWLEDNLSEGIREWWDLKPGAPKPKANQQKQDNGRGLVLPGYKYLGPFNGLDKGEPVNAADAAALEHDKAYDQQLQAGDNPYLRYNHADAEFQERLQEDTSFGGNLGRAVFQAKKRVLEPLGLVESPVKTAPGKKRPVEPSPQRSPDSSTGIGKKGQQPAKKRLNFGQTGDSESVPDPQPIGEPPAAPSGVGPNTMAAGGGAPMADNNEGADGVGSSSGNWHCDSTWLGDRVITTSTRTWALPTYNNHLYKQISNGTSGGSTNDNTYFGYSTPWGYFDFNRFHCHFSPRDWQRLINNNWGFRPKRLNFKLFNIQVKEVTQNEGTKTIANNLTSTIQVFTDSEYQLPYVLGSAHQGCLPPFPADVFMIPQYGYLTLNNGSQAVGRSSFYCLEYFPSQMLRTGNNFEFSYNFEDVPFHSSYAHSQSLDRLMNPLIDQYLYYLSRTQSTGGTAGTQQLLFSQAGPNNMSAQAKNWLPGPCYRQQRVSTTLSQNNNSNFAWTGATKYHLNGRDSLVNPGVAMATHKDDEERFFPSSGVLMFGKQGAGKDNVDYSSVMLTSEEEIKTTNPVATEQYGVVADNLQQQNAAPIVGAVNSQGALPGMVWQNRDVYLQGPIWAKIPHTDGNFHPSPLMGGFGLKHPPPQILIKNTPVPADPPTTFNQAKLASFITQYSTGQVSVEIEWELQKENSKRWNPEIQYTSNYYKSTNVDFAVNTEGTYSEPRPIGTRYLTRNL

SEQ ID NO: 41 - protein, 736 aa, Artificial Sequence
  VP1 Capsid
MAADGYLPDWLEDNLSEGIREWWALQPGAPKPKANQQHQDNARGLVLPGYKYLGPGNGLDKGEPVNAADAAALEHDKAYDQQLKAGDNPYLKYNHADAEFQERLKEDTSFGGNLGRAVFQAKKRLLEPLGLVEEAAKTAPGKKRPVDQSPQEPDSSSGVGKSGKQPARKRLNFGQTGDSESVPDPQPLGEPPAAPTSLGSNTMASGGGAPMADNNEGADGVGNSSGNWHCDSQWLGDRVITTSTRTWALPTYNNHLYKQISSQSGASNDNHYFGYSTPWGYFDFNRFHCHFSPRDWQRLINNNWGFRPKKLSFKLFNIQVKEVTQNDGTTTIANNLTSTVQVFTDSEYQLPYVLGSAHQGCLPPFPADVFMVPQYGYLTLNNGSQAVGRSSFYCLEYFPSQMLRTGNNFQFSYTFEDVPFHSSYAHSQSLDRLMNPLIDQYLYYLNRTQGTTSGTTNQSRLLFSQAGPQSMSLQARNWLPGPCYRQQRLSKTANDNNNSNFPWTAASKYHLNGRDSLVNPGPAMASHKDDEEKFFPMHGNLIFGKEGTTASNAELDNVMITDEEEIRTTNPVATEQYGTVANNLQSSNTAPTTRTVNDQGALPGMVWQDRDVYLQGPIWAKIPHTDGHFHPSPLMGGFGLKHPPPQIMIKNTPVPANPPTTFSPAKFASFITQYSTGQVSVEIEWELQKENSKRWNPEIQYTSNYNKSVNVDFTVDTNGVYSEPRPIGTRYLTRPL

SEQ ID NO: 42 - DNA, 264 bp, Homo sapiens
aaggtcgggcaggaagagggcctatttcccatgattccttcatatttgcatatacgatacaaggctgttagagagataattagaattaatttgactgtaaacacaaagatattagtacaaaatacgtgacgtagaaagtaataatttcttgggtagtttgcagttttaaaattatgttttaaaatggactatcatatgcttaccgtaacttgaaagtatttcgatttcttggctttatatatcttgtggaaaggacgaaacacc

SEQ ID NO: 43 - DNA, 313 bp, Mus musculus
atccgacgccgccatctctaggcccgcgccggccccctcgcacagacttgtgggagaagctcggctactcccctgccccggttaatttgcatataatatttcctagtaactatagaggcttaatgtgcgataaaagacagataatctgttctttttaatactagctacattttacatgataggcttggatttctataagagatacaaatactaaattattattttaaaaaacagcacaaaaggaaactcaccctaactgtaaagtaattgtgtgttttgagactataaatatcccttggagaaaagccttgtt

SEQ ID NO: 44 - DNA, 215 bp, Homo sapiens
gaacgctgacgtcatcaacccgctccaaggaatcgcgggcccagtgtcactaggcgggaacacccagcgcgcgtgcgccctggcaggaagatggctgtgagggacaggggagtggcgccctgcaatatttgcatgtcgctatgtgttctgggaaatcaccataaacgtgaaatgtctttggatttgggaatcgtataagaactgtatgagaccac

SEQ ID NO: 45 - DNA, 190 bp, Homo sapiens
agctctagcttgaattggtgccactgttcggcatcgttgtgtttcgatctctacaatttcgttacggtagcctctccagctctagcctagctatttgcatgtcgctatgtgttctgggaaatcaccataaacgtgaaatgtctttggatttgggaatcttataagttctgtatgagaccactctttccca